European Patent Application EP 4 755 378 A1, published June 10, 2026. Title: DYRK2 INHIBITORS FOR TREATING TUMOURS WITH THE HYPERACTIVE MAPK/ERK PATHWAY. Applicant: Universidad de Córdoba. Application ES. The sequence listing filed with the application follows.

SEQUENCE LISTING (10 sequences)

SEQ ID NO: 1 - DNA, 45 bp, synthetic construct
  source 1..45: mol_type = other DNA
cccaggccaagggcccccgggaggccccttgcctcatacggaatg

SEQ ID NO: 2 - DNA, 45 bp, synthetic construct
  source 1..45: mol_type = other DNA
ggctgtccattccgtatgaggcaaggggcctcccgggggcccttg

SEQ ID NO: 3 - DNA, 45 bp, synthetic construct; identical to SEQ ID NO: 1
  source 1..45: mol_type = other DNA

SEQ ID NO: 4 - DNA, 45 bp, synthetic construct; identical to SEQ ID NO: 2
  source 1..45: mol_type = other DNA

SEQ ID NO: 5 - DNA, 43 bp, synthetic construct
  source 1..43: mol_type = other DNA
ggggtcagcgggcagctcatcgacgccatggccaacgccttcg

SEQ ID NO: 6 - DNA, 43 bp, synthetic construct
  source 1..43: mol_type = other DNA
gtaggaccttgtgcccacgaaggcgttggccatggcgtcgatg

SEQ ID NO: 7 - DNA, 22 bp, synthetic construct
  source 1..22: mol_type = other DNA
aacgagaccgatcctcatcagc

SEQ ID NO: 8 - DNA, 23 bp, synthetic construct
  source 1..23: mol_type = other DNA
ggtagcagacaaacctgtggttg

SEQ ID NO: 9 - DNA, 24 bp, synthetic construct
  source 1..24: mol_type = other DNA
cattatgctgaggatttggaaagg

SEQ ID NO: 10 - DNA, 22 bp, synthetic construct
  source 1..22: mol_type = other DNA
cttgagcacacagagggctaca